European Patent Specification EP 4 017 973 B1, published June 10, 2026. Title: Biosynthesis of Eriodictyol. Applicant: Conagen Inc. The sequence listing filed with the application follows.

SEQUENCE LISTING (20 sequences)

SEQ ID NO: 1 - DNA, 1512 bp, Artificial Sequence
  SsPvcC-M196Y mutant
atgacgggcgccgaatatctggattcgctgcgtgatggccgtgccgtctatattcacggcgaacgcgtccgcgatgtcaccgcgcatccggccttccgtaacagcgcgcgtagtctggcgcagctgtatgatgtgctgcatgaaccggattcgcgtggcgttctgagcgtcccgaccgataccggtaatggcggttttacgcacccgtttttcaaaaccgcgcgtagcgccggtgatctggtggcagcccgcgatgcaattgtggcctggcagcgtcttgtttacggttggatgggtcgtacgccggattataaagcagcattcttcggtacgcttgaagccaacgccgatttctatggcccgttccgtgataacgcactggcatggtatcgtcgtgcacaggaacgcgtgttgtatttcaaccatgcgatcgtgcatccgccggtcgatcgcgatcgcccggccgatcgcacggcggatgtgtgcgtccacgtggaagaagaaacggatgccggccttgttgtttcgggtgcgaaagttgtcgcgaccagcagcgccctgacgaatgccaatctgattgcacactacggcttaccgctgcgtgataaacgctttggcgccatgttcaccgtgccgatggatagcccgggcctgaaactgttctgtcgtaccagttatgaaatgcatgccgcggtcttaggctcgccgtttgattacccgttaagcagccgccttgatgaaaatgattcaatcatggttcttgatcgtgttttagtgccgtgggaaaacgtgtttatgtatgatgccgccagcgcgaacgcgtttgcgacccgcagcggtttcctggaacgttttacctttcatggctgtacgcgcttagcggtgaaactggattttattgccggttgcctgctgaaagcagttgaagtgaccggcaccagcggcttccgtggtgtgcaggcccagattggcgaagttttaaactggcgcgatatgttttggggtatgtcagatgcaatggcgaaatcgccgacggattggcacaatggtgcggtccagccgaatctgaactatggcctggcctaccgcaccttcatgggcattggttacccgcgtatccgtgaaatcattcagcagaccattggctcgggtctgatttatttaaatagtcacgcaagcgattggaaaaatccggaagttcgtccgtacttagatcgctacctgcgcggtagtcgtggtgttgaagcgatcgatcgcgttaaactgcttaaactgctgtgggattgcgtgggcacggaatttgcgggccgtcacgaactttatgaacgcaattacggtggcgatcatgaaggtattcgcgtgcagaccctgttgagttatcaggcgcgcggtcaggcggatgcgcttaaaggctttgccgatcagtgtatgtcagaatacgatctggatggctggacccgcccggatttattcggtccaggtgatttacctagaccagctactggagcgtaa

SEQ ID NO: 2 - protein, 503 aa, Artificial Sequence
  SsPvcC-M196Y mutant
MTGAEYLDSLRDGRAVYIHGERVRDVTAHPAFRNSARSLAQLYDVLHEPDSRGVLSVPTDTGNGGFTHPFFKTARSAGDLVAARDAIVAWQRLVYGWMGRTPDYKAAFFGTLEANADFYGPFRDNALAWYRRAQERVLYFNHAIVHPPVDRDRPADRTADVCVHVEEETDAGLVVSGAKVVATSSALTNANLIAHYGLPLRDKRFGAMFTVPMDSPGLKLFCRTSYEMHAAVLGSPFDYPLSSRLDENDSIMVLDRVLVPWENVFMYDAASANAFATRSGFLERFTFHGCTRLAVKLDFIAGCLLKAVEVTGTSGFRGVQAQIGEVLNWRDMFWGMSDAMAKSPTDWHNGAVQPNLNYGLAYRTFMGIGYPRIREIIQQTIGSGLIYLNSHASDWKNPEVRPYLDRYLRGSRGVEAIDRVKLLKLLWDCVGTEFAGRHELYERNYGGDHEGIRVQTLLSYQARGQADALKGFADQCMSEYDLDGWTRPDLFGPGDLPRPATGA

SEQ ID NO: 3 - DNA, 1563 bp, Artificial Sequence
  SsPvcC-M196Y-Tag
atgacgaccgctagtggtaccaatgcagatgtccagaatggcgtccgcccgatgacgggcgccgaatatctggattcgctgcgtgatggccgtgccgtctatattcacggcgaacgcgtccgcgatgtcaccgcgcatccggccttccgtaacagcgcgcgtagtctggcgcagctgtatgatgtgctgcatgaaccggattcgcgtggcgttctgagcgtcccgaccgataccggtaatggcggttttacgcacccgtttttcaaaaccgcgcgtagcgccggtgatctggtggcagcccgcgatgcaattgtggcctggcagcgtcttgtttacggttggatgggtcgtacgccggattataaagcagcattcttcggtacgcttgaagccaacgccgatttctatggcccgttccgtgataacgcactggcatggtatcgtcgtgcacaggaacgcgtgttgtatttcaaccatgcgatcgtgcatccgccggtcgatcgcgatcgcccggccgatcgcacggcggatgtgtgcgtccacgtggaagaagaaacggatgccggccttgttgtttcgggtgcgaaagttgtcgcgaccagcagcgccctgacgaatgccaatctgattgcacactacggcttaccgctgcgtgataaacgctttggcgccatgttcaccgtgccgatggatagcccgggcctgaaactgttctgtcgtaccagttatgaaatgcatgccgcggtcttaggctcgccgtttgattacccgttaagcagccgccttgatgaaaatgattcaatcatggttcttgatcgtgttttagtgccgtgggaaaacgtgtttatgtatgatgccgccagcgcgaacgcgtttgcgacccgcagcggtttcctggaacgttttacctttcatggctgtacgcgcttagcggtgaaactggattttattgccggttgcctgctgaaagcagttgaagtgaccggcaccagcggcttccgtggtgtgcaggcccagattggcgaagttttaaactggcgcgatatgttttggggtatgtcagatgcaatggcgaaatcgccgacggattggcacaatggtgcggtccagccgaatctgaactatggcctggcctaccgcaccttcatgggcattggttacccgcgtatccgtgaaatcattcagcagaccattggctcgggtctgatttatttaaatagtcacgcaagcgattggaaaaatccggaagttcgtccgtacttagatcgctacctgcgcggtagtcgtggtgttgaagcgatcgatcgcgttaaactgcttaaactgctgtgggattgcgtgggcacggaatttgcgggccgtcacgaactttatgaacgcaattacggtggcgatcatgaaggtattcgcgtgcagaccctgttgagttatcaggcgcgcggtcaggcggatgcgcttaaaggctttgccgatcagtgtatgtcagaatacgatctggatggctggacccgcccggatttattcggtccaggtgatttacctagaccagctactggagcgtaa

SEQ ID NO: 4 - protein, 520 aa, Artificial Sequence
  SsPvcC-M196Y-Tag mutant
MTTASGTNADVQNGVRPMTGAEYLDSLRDGRAVYIHGERVRDVTAHPAFRNSARSLAQLYDVLHEPDSRGVLSVPTDTGNGGFTHPFFKTARSAGDLVAARDAIVAWQRLVYGWMGRTPDYKAAFFGTLEANADFYGPFRDNALAWYRRAQERVLYFNHAIVHPPVDRDRPADRTADVCVHVEEETDAGLVVSGAKVVATSSALTNANLIAHYGLPLRDKRFGAMFTVPMDSPGLKLFCRTSYEMHAAVLGSPFDYPLSSRLDENDSIMVLDRVLVPWENVFMYDAASANAFATRSGFLERFTFHGCTRLAVKLDFIAGCLLKAVEVTGTSGFRGVQAQIGEVLNWRDMFWGMSDAMAKSPTDWHNGAVQPNLNYGLAYRTFMGIGYPRIREIIQQTIGSGLIYLNSHASDWKNPEVRPYLDRYLRGSRGVEAIDRVKLLKLLWDCVGTEFAGRHELYERNYGGDHEGIRVQTLLSYQARGQADALKGFADQCMSEYDLDGWTRPDLFGPGDLPRPATGA

SEQ ID NO: 5 - DNA, 1563 bp, Artificial Sequence
  SsPvcC-G315H+Tag mutant
atgacgaccgctagtggtaccaatgcagatgtccagaatggcgtccgcccgatgacgggcgccgaatatctggattcgctgcgtgatggccgtgccgtctatattcacggcgaacgcgtccgcgatgtcaccgcgcatccggccttccgtaacagcgcgcgtagtctggcgcagctgtatgatgtgctgcatgaaccggattcgcgtggcgttctgagcgtcccgaccgataccggtaatggcggttttacgcacccgtttttcaaaaccgcgcgtagcgccggtgatctggtggcagcccgcgatgcaattgtggcctggcagcgtcttgtttacggttggatgggtcgtacgccggattataaagcagcattcttcggtacgcttgaagccaacgccgatttctatggcccgttccgtgataacgcactggcatggtatcgtcgtgcacaggaacgcgtgttgtatttcaaccatgcgatcgtgcatccgccggtcgatcgcgatcgcccggccgatcgcacggcggatgtgtgcgtccacgtggaagaagaaacggatgccggccttgttgtttcgggtgcgaaagttgtcgcgaccagcagcgccctgacgaatgccaatctgattgcacacatgggcttaccgctgcgtgataaacgctttggcgccatgttcaccgtgccgatggatagcccgggcctgaaactgttctgtcgtaccagttatgaaatgcatgccgcggtcttaggctcgccgtttgattacccgttaagcagccgccttgatgaaaatgattcaatcatggttcttgatcgtgttttagtgccgtgggaaaacgtgtttatgtatgatgccgccagcgcgaacgcgtttgcgacccgcagcggtttcctggaacgttttacctttcatggctgtacgcgcttagcggtgaaactggattttattgccggttgcctgctgaaagcagttgaagtgaccggcaccagccacttccgtggtgtgcaggcccagattggcgaagttttaaactggcgcgatatgttttggggtatgtcagatgcaatggcgaaatcgccgacggattggcacaatggtgcggtccagccgaatctgaactatggcctggcctaccgcaccttcatgggcattggttacccgcgtatccgtgaaatcattcagcagaccattggctcgggtctgatttatttaaatagtcacgcaagcgattggaaaaatccggaagttcgtccgtacttagatcgctacctgcgcggtagtcgtggtgttgaagcgatcgatcgcgttaaactgcttaaactgctgtgggattgcgtgggcacggaatttgcgggccgtcacgaactttatgaacgcaattacggtggcgatcatgaaggtattcgcgtgcagaccctgttgagttatcaggcgcgcggtcaggcggatgcgcttaaaggctttgccgatcagtgtatgtcagaatacgatctggatggctggacccgcccggatttattcggtccaggtgatttacctagaccagctactggagcgtaa

SEQ ID NO: 6 - protein, 520 aa, Artificial Sequence
  SsPvcC-G315H+Tag mutant
MTTASGTNADVQNGVRPMTGAEYLDSLRDGRAVYIHGERVRDVTAHPAFRNSARSLAQLYDVLHEPDSRGVLSVPTDTGNGGFTHPFFKTARSAGDLVAARDAIVAWQRLVYGWMGRTPDYKAAFFGTLEANADFYGPFRDNALAWYRRAQERVLYFNHAIVHPPVDRDRPADRTADVCVHVEEETDAGLVVSGAKVVATSSALTNANLIAHMGLPLRDKRFGAMFTVPMDSPGLKLFCRTSYEMHAAVLGSPFDYPLSSRLDENDSIMVLDRVLVPWENVFMYDAASANAFATRSGFLERFTFHGCTRLAVKLDFIAGCLLKAVEVTGTSHFRGVQAQIGEVLNWRDMFWGMSDAMAKSPTDWHNGAVQPNLNYGLAYRTFMGIGYPRIREIIQQTIGSGLIYLNSHASDWKNPEVRPYLDRYLRGSRGVEAIDRVKLLKLLWDCVGTEFAGRHELYERNYGGDHEGIRVQTLLSYQARGQADALKGFADQCMSEYDLDGWTRPDLFGPGDLPRPATGA

SEQ ID NO: 7 - DNA, 1563 bp, Artificial Sequence
  SsPvcC-D214N+Tag mutant
atgacgaccgctagtggtaccaatgcagatgtccagaatggcgtccgcccgatgacgggcgccgaatatctggattcgctgcgtgatggccgtgccgtctatattcacggcgaacgcgtccgcgatgtcaccgcgcatccggccttccgtaacagcgcgcgtagtctggcgcagctgtatgatgtgctgcatgaaccggattcgcgtggcgttctgagcgtcccgaccgataccggtaatggcggttttacgcacccgtttttcaaaaccgcgcgtagcgccggtgatctggtggcagcccgcgatgcaattgtggcctggcagcgtcttgtttacggttggatgggtcgtacgccggattataaagcagcattcttcggtacgcttgaagccaacgccgatttctatggcccgttccgtgataacgcactggcatggtatcgtcgtgcacaggaacgcgtgttgtatttcaaccatgcgatcgtgcatccgccggtcgatcgcgatcgcccggccgatcgcacggcggatgtgtgcgtccacgtggaagaagaaacggatgccggccttgttgtttcgggtgcgaaagttgtcgcgaccagcagcgccctgacgaatgccaatctgattgcacacatgggcttaccgctgcgtgataaacgctttggcgccatgttcaccgtgccgatgaatagcccgggcctgaaactgttctgtcgtaccagttatgaaatgcatgccgcggtcttaggctcgccgtttgattacccgttaagcagccgccttgatgaaaatgattcaatcatggttcttgatcgtgttttagtgccgtgggaaaacgtgtttatgtatgatgccgccagcgcgaacgcgtttgcgacccgcagcggtttcctggaacgttttacctttcatggctgtacgcgcttagcggtgaaactggattttattgccggttgcctgctgaaagcagttgaagtgaccggcaccagccatttccgtggtgtgcaggcccagattggcgaagttttaaactggcgcgatatgttttggggtatgtcagatgcaatggcgaaatcgccgacggattggcacaatggtgcggtccagccgaatctgaactatggcctggcctaccgcaccttcatgggcattggttacccgcgtatccgtgaaatcattcagcagaccattggctcgggtctgatttatttaaatagtcacgcaagcgattggaaaaatccggaagttcgtccgtacttagatcgctacctgcgcggtagtcgtggtgttgaagcgatcgatcgcgttaaactgcttaaactgctgtgggattgcgtgggcacggaatttgcgggccgtcacgaactttatgaacgcaattacggtggcgatcatgaaggtattcgcgtgcagaccctgttgagttatcaggcgcgcggtcaggcggatgcgcttaaaggctttgccgatcagtgtatgtcagaatacgatctggatggctggacccgcccggatttattcggtccaggtgatttacctagaccagctactggagcgtaa

SEQ ID NO: 8 - protein, 520 aa, Artificial Sequence
  SsPvcC-D214N+Tag mutant
MTTASGTNADVQNGVRPMTGAEYLDSLRDGRAVYIHGERVRDVTAHPAFRNSARSLAQLYDVLHEPDSRGVLSVPTDTGNGGFTHPFFKTARSAGDLVAARDAIVAWQRLVYGWMGRTPDYKAAFFGTLEANADFYGPFRDNALAWYRRAQERVLYFNHAIVHPPVDRDRPADRTADVCVHVEEETDAGLVVSGAKVVATSSALTNANLIAHMGLPLRDKRFGAMFTVPMNSPGLKLFCRTSYEMHAAVLGSPFDYPLSSRLDENDSIMVLDRVLVPWENVFMYDAASANAFATRSGFLERFTFHGCTRLAVKLDFIAGCLLKAVEVTGTSGFRGVQAQIGEVLNWRDMFWGMSDAMAKSPTDWHNGAVQPNLNYGLAYRTFMGIGYPRIREIIQQTIGSGLIYLNSHASDWKNPEVRPYLDRYLRGSRGVEAIDRVKLLKLLWDCVGTEFAGRHELYERNYGGDHEGIRVQTLLSYQARGQADALKGFADQCMSEYDLDGWTRPDLFGPGDLPRPATGA

SEQ ID NO: 9 - DNA, 1563 bp, Artificial Sequence
  SsPvcC+Tag
atgacgaccgctagtggtaccaatgcagatgtccagaatggcgtccgcccgatgacgggcgccgaatatctggattcgctgcgtgatggccgtgccgtctatattcacggcgaacgcgtccgcgatgtcaccgcgcatccggccttccgtaacagcgcgcgtagtctggcgcagctgtatgatgtgctgcatgaaccggattcgcgtggcgttctgagcgtcccgaccgataccggtaatggcggttttacgcacccgtttttcaaaaccgcgcgtagcgccggtgatctggtggcagcccgcgatgcaattgtggcctggcagcgtcttgtttacggttggatgggtcgtacgccggattataaagcagcattcttcggtacgcttgaagccaacgccgatttctatggcccgttccgtgataacgcactggcatggtatcgtcgtgcacaggaacgcgtgttgtatttcaaccatgcgatcgtgcatccgccggtcgatcgcgatcgcccggccgatcgcacggcggatgtgtgcgtccacgtggaagaagaaacggatgccggccttgttgtttcgggtgcgaaagttgtcgcgaccagcagcgccctgacgaatgccaatctgattgcacacatgggcttaccgctgcgtgataaacgctttggcgccatgttcaccgtgccgatggatagcccgggcctgaaactgttctgtcgtaccagttatgaaatgcatgccgcggtcttaggctcgccgtttgattacccgttaagcagccgccttgatgaaaatgattcaatcatggttcttgatcgtgttttagtgccgtgggaaaacgtgtttatgtatgatgccgccagcgcgaacgcgtttgcgacccgcagcggtttcctggaacgttttacctttcatggctgtacgcgcttagcggtgaaactggattttattgccggttgcctgctgaaagcagttgaagtgaccggcaccagcggcttccgtggtgtgcaggcccagattggcgaagttttaaactggcgcgatatgttttggggtatgtcagatgcaatggcgaaatcgccgacggattggcacaatggtgcggtccagccgaatctgaactatggcctggcctaccgcaccttcatgggcattggttacccgcgtatccgtgaaatcattcagcagaccattggctcgggtctgatttatttaaatagtcacgcaagcgattggaaaaatccggaagttcgtccgtacttagatcgctacctgcgcggtagtcgtggtgttgaagcgatcgatcgcgttaaactgcttaaactgctgtgggattgcgtgggcacggaatttgcgggccgtcacgaactttatgaacgcaattacggtggcgatcatgaaggtattcgcgtgcagaccctgttgagttatcaggcgcgcggtcaggcggatgcgcttaaaggctttgccgatcagtgtatgtcagaatacgatctggatggctggacccgcccggatttattcggtccaggtgatttacctagaccagctactggagcgtaa

SEQ ID NO: 10 - protein, 520 aa, Artificial Sequence
  SsPvcC+Tag
MTTASGTNADVQNGVRPMTGAEYLDSLRDGRAVYIHGERVRDVTAHPAFRNSARSLAQLYDVLHEPDSRGVLSVPTDTGNGGFTHPFFKTARSAGDLVAARDAIVAWQRLVYGWMGRTPDYKAAFFGTLEANADFYGPFRDNALAWYRRAQERVLYFNHAIVHPPVDRDRPADRTADVCVHVEEETDAGLVVSGAKVVATSSALTNANLIAHMGLPLRDKRFGAMFTVPMDSPGLKLFCRTSYEMHAAVLGSPFDYPLSSRLDENDSIMVLDRVLVPWENVFMYDAASANAFATRSGFLERFTFHGCTRLAVKLDFIAGCLLKAVEVTGTSGFRGVQAQIGEVLNWRDMFWGMSDAMAKSPTDWHNGAVQPNLNYGLAYRTFMGIGYPRIREIIQQTIGSGLIYLNSHASDWKNPEVRPYLDRYLRGSRGVEAIDRVKLLKLLWDCVGTEFAGRHELYERNYGGDHEGIRVQTLLSYQARGQADALKGFADQCMSEYDLDGWTRPDLFGPGDLPRPATGA

SEQ ID NO: 11 - DNA, 1512 bp, Streptomyces sclerotialus
atgacgggcgccgaatatctggattcgctgcgtgatggccgtgccgtctatattcacggcgaacgcgtccgcgatgtcaccgcgcatccggccttccgtaacagcgcgcgtagtctggcgcagctgtatgatgtgctgcatgaaccggattcgcgtggcgttctgagcgtcccgaccgataccggtaatggcggttttacgcacccgtttttcaaaaccgcgcgtagcgccggtgatctggtggcagcccgcgatgcaattgtggcctggcagcgtcttgtttacggttggatgggtcgtacgccggattataaagcagcattcttcggtacgcttgaagccaacgccgatttctatggcccgttccgtgataacgcactggcatggtatcgtcgtgcacaggaacgcgtgttgtatttcaaccatgcgatcgtgcatccgccggtcgatcgcgatcgcccggccgatcgcacggcggatgtgtgcgtccacgtggaagaagaaacggatgccggccttgttgtttcgggtgcgaaagttgtcgcgaccagcagcgccctgacgaatgccaatctgattgcacacatgggcttaccgctgcgtgataaacgctttggcgccatgttcaccgtgccgatggatagcccgggcctgaaactgttctgtcgtaccagttatgaaatgcatgccgcggtcttaggctcgccgtttgattacccgttaagcagccgccttgatgaaaatgattcaatcatggttcttgatcgtgttttagtgccgtgggaaaacgtgtttatgtatgatgccgccagcgcgaacgcgtttgcgacccgcagcggtttcctggaacgttttacctttcatggctgtacgcgcttagcggtgaaactggattttattgccggttgcctgctgaaagcagttgaagtgaccggcaccagcggcttccgtggtgtgcaggcccagattggcgaagttttaaactggcgcgatatgttttggggtatgtcagatgcaatggcgaaatcgccgacggattggcacaatggtgcggtccagccgaatctgaactatggcctggcctaccgcaccttcatgggcattggttacccgcgtatccgtgaaatcattcagcagaccattggctcgggtctgatttatttaaatagtcacgcaagcgattggaaaaatccggaagttcgtccgtacttagatcgctacctgcgcggtagtcgtggtgttgaagcgatcgatcgcgttaaactgcttaaactgctgtgggattgcgtgggcacggaatttgcgggccgtcacgaactttatgaacgcaattacggtggcgatcatgaaggtattcgcgtgcagaccctgttgagttatcaggcgcgcggtcaggcggatgcgcttaaaggctttgccgatcagtgtatgtcagaatacgatctggatggctggacccgcccggatttattcggtccaggtgatttacctagaccagctactggagcgtaa

SEQ ID NO: 12 - protein, 503 aa, Streptomyces sclerotialus
MTGAEYLDSLRDGRAVYIHGERVRDVTAHPAFRNSARSLAQLYDVLHEPDSRGVLSVPTDTGNGGFTHPFFKTARSAGDLVAARDAIVAWQRLVYGWMGRTPDYKAAFFGTLEANADFYGPFRDNALAWYRRAQERVLYFNHAIVHPPVDRDRPADRTADVCVHVEEETDAGLVVSGAKVVATSSALTNANLIAHMGLPLRDKRFGAMFTVPMDSPGLKLFCRTSYEMHAAVLGSPFDYPLSSRLDENDSIMVLDRVLVPWENVFMYDAASANAFATRSGFLERFTFHGCTRLAVKLDFIAGCLLKAVEVTGTSGFRGVQAQIGEVLNWRDMFWGMSDAMAKSPTDWHNGAVQPNLNYGLAYRTFMGIGYPRIREIIQQTIGSGLIYLNSHASDWKNPEVRPYLDRYLRGSRGVEAIDRVKLLKLLWDCVGTEFAGRHELYERNYGGDHEGIRVQTLLSYQARGQADALKGFADQCMSEYDLDGWTRPDLFGPGDLPRPATGA

SEQ ID NO: 13 - DNA, 510 bp, Saccharothrix espanaensis
atgatgaccgtttatgatagcgcactgacaatggaagaaaccaccctgcgtgatgcaatgagccgttttgcaaccggtgttagcgttgttaccgttggtggtgaacatacacatggtatgaccgcaaatgcctttacctgtgttagcctggatccgcctctggttctgtgttgtgttgcacgtaaagcaaccatgcatgcagcaattgaaggtgcacgtcgttttgcagttagcgttatgggtggtgatcaagaacgtaccgcacgttattttgcagataaacgtcgtccgcgtggtcgtgcacagtttgatgttgttgattggcagcctggtccgcatacaggtgcaccgctgctgagcggtgcgctggcatggctggaatgtgaagttgcacagtggcatgaaggtggcgatcataccatttttctgggtcgtgttctgggttgtcgtcgtggtccggatagtccggcactgctgttttatggtagcgattttcatcagatccgctaa

SEQ ID NO: 14 - protein, 169 aa, Saccharothrix espanaensis
MMTVYDSALTMEETTLRDAMSRFATGVSVVTVGGEHTHGMTANAFTCVSLDPPLVLCCVARKATMHAAIEGARRFAVSVMGGDQERTARYFADKRRPRGRAQFDVVDWQPGPHTGAPLLSGALAWLECEVAQWHEGGDHTIFLGRVLGCRRGPDSPALLFYGSDFHQIR

SEQ ID NO: 15 - DNA, 561 bp, Pseudomonas fluorescens
atgaatgcagcaaccgaaaccaaagttcatgatctgctggatgccgaaggtcgtgatgttcgtgatgcacgtgaactgcgtaatgttctgggtcagtttgcaaccggtgttaccgttattaccacccgtaccgcagatggtcgtaatgttggtgtgaccgcaaatagctttagcagcctgagcctgagtccggcactggttctgtggtcactggcacgtaccgcaccgagcctgaaagttttttgtagcgcaagccattttgccattaatgtgctgggtgcacatcagctgcatctgagcgaacagtttgcacgtgccgcagcagataaatttgccggtgttgcacatagttatggtaaagcgggtgcaccggttctggatgatgttgttgcagttctggtttgccgtaatgttacccagtatgaaggtggtgatcatctgatttttatcggcgaaattgagcagtatcgttatagcggtgcagaaccgctggtttttcatgcaggtcagtatcgtggtctgggtagcaatcgtgcagaaagcgttctgaaacatgaataa

SEQ ID NO: 16 - protein, 186 aa, Pseudomonas fluorescens
MNAATETKVHDLLDAEGRDVRDARELRNVLGQFATGVTVITTRTADGRNVGVTANSFSSLSLSPALVLWSLARTAPSLKVFCSASHFAINVLGAHQLHLSEQFARAAADKFAGVAHSYGKAGAPVLDDVVAVLVCRNVTQYEGGDHLIFIGEIEQYRYSGAEPLVFHAGQYRGLGSNRAESVLKHE

SEQ ID NO: 17 - DNA, 513 bp, Escherichia coli
atgcaattagatgaacaacgcctgcgctttcgtgacgcaatggccagcctgtcggcagcggtaaatattatcaccaccgagggcgacgccggacaatgcgggattacggcaacggccgtctgctcggtcacggatacaccaccatcgctgatggtgtgcattaacgccaacagtgcgatgaacccggtttttcagggcaacggtaagttgtgcgtcaacgtcctcaaccatgagcaggaactgatggcacgccacttcgcgggcatgacaggcatggcgatggaagagcgttttagcctctcatgctggcaaaaaggtccgctggcgcagccggtgctaaaaggttcgctggccagtcttgaaggtgagatccgcgatgtgcaggcaattggcacacatctggtgtatctggtggagattaaaaacatcatcctcagtgcagaaggtcacggacttatctactttaaacgccgtttccatccggtgatgctggaaatggaagctgcgatttaa

SEQ ID NO: 18 - protein, 170 aa, Escherichia coli
MQLDEQRLRFRDAMASLSAAVNIITTEGDAGQCGITATAVCSVTDTPPSLMVCINANSAMNPVFQGNGKLCVNVLNHEQELMARHFAGMTGMAMEERFSLSCWQKGPLAQPVLKGSLASLEGEIRDVQAIGTHLVYLVEIKNIILSAEGHGLIYFKRRFHPVMLEMEAAI

SEQ ID NO: 19 - DNA, 51 bp, Artificial Sequence
  N-terminal tag
atgacgaccgctagtggtaccaatgcagatgtccagaatggcgtccgcccg

SEQ ID NO: 20 - protein, 17 aa, Artificial Sequence
  N-terminal tag
MTTASGTNADVQNGVRP